European Patent Application EP 4 585 923 A1, published July 16, 2025. Title: 诊断MIDD的方法和试剂盒. Applicant: 华东理工大学. The sequence listing filed with the application follows.

SEQUENCE LISTING (7 sequences)

SEQ ID NO: 1 - protein, 258 aa, synthetic construct
MIVLPRRLSDEVADRVRALIDEKNLEAGMKLPAERQLAMQLGVSRNSLREALAKLVSEGVLLSRRGGGTFIRWRHDTWSEQNIVQPLKTLMADDPDYSFDILEARYAIEASTAWHAAMRATPGDKEKIQLCFEATLSEDPDIASQADVRFHLAIAEASHNIVLLQTMRGFFDVLQSSVKHSRQRMYLVPPVFSQLTEQHQAVIDAIFAGDADGARKAMMAHLSFVHTTMKRFDEDQARHARITRLPGEHNEHSREKNA

SEQ ID NO: 2 - protein, 423 aa, synthetic construct
MEQNIVQPLKTLMADDPDYSFDILEARYAIEASTAWHAAMRATPGDKEKIQLCFEATLSEDPDIASQADVRFHLAIAEASHNIVLLQTMRGFFDVLQSSVKHSRQRMYNSDNVYIMADKQKNGIKANFKIRHNVEDGSVQLADHYQQNTPIGDGPVLLPDNHYLSFQSVLSKDPNEKRDHMVLLEFVTAAGITLGMDELYNVDGGSGGTGSKGEELFTGVVPILVELDGDVNGHKFSVSGEGEGDATYGKLTLKLICTTGKLPVPWPTLVTTLGYGLKCFARYPDHMKQHDFFKSAMPEGYVQERTIFFKDDGNYKTRAEVKFEGDTLVNRIELKGIDFKEDGNILGHKLEYNFDVFSQLTEQHQAVIDAIFAGDADGARKAMMAHLSFVHTTMKRFDEDQARHARITRLPGEHNEHSREKNA

SEQ ID NO: 3 - protein, 423 aa, synthetic construct
MEQNIVQPLKTLMADDPDYSFDILEARYAIEASTAWHAAMRATPGDKEKIQLCFEATLSEDPDIASQADVRFHLAIAEASHNIVLLQTMRGFFDVLQSSVKHSRQRLYNSDNVYIMADKQKNGIKANFKIRHNVEDGSVQLADHYQQNTPIGDGPVLLPDNHYLSFQSVLSKDPNEKRDHMVLLEFVTAAGITLGMDELYNVDGGSGGTGSKGEELFTGVVPILVELDGDVNGHKFSVSGEGEGDATYGKLTLKLICTTGKLPVPWPTLVTTLGYGLKCFARYPDHMKQHDFFKSAMPEGYVQERTIFFKDDGNYKTRAEVKFEGDTLVNRIELKGIDFKEDGNILGHKLEYNHDVFSQLTEQHQAVIDAIFAGDADGARKAMMAHLSFVHTTMKRFDEDQARHARITRLPGEHNEHSREKNA

SEQ ID NO: 4 - protein, 246 aa, synthetic construct
YNSDNVYIMADKQKNGIKANFKIRHNVEDGSVQLADHYQQNTPIGDGPVLLPDNHYLSFQSVLSKDPNEKRDHMVLLEFVTAAGITLGMDELYNVDGGSGGTGSKGEELFTGVVPILVELDGDVNGHKFSVSGEGEGDATYGKLTLKLICTTGKLPVPWPTLVTTLGYGLKCFARYPDHMKQHDFFKSAMPEGYVQERTIFFKDDGNYKTRAEVKFEGDTLVNRIELKGIDFKEDGNILGHKLEYN

SEQ ID NO: 5 - protein, 241 aa, synthetic construct
NVYIKADKQKNGIKANFKIRHNIEDGGVQLAYHYQQNTPIGDGPVLLPDNHYLSVQSILSKDPNEKRDHMVLLEFVTAAGITLGMDELYKGGTGGSMVSKGEELFTGVVPIQVELDGDVNGHKFSVSGEGEGDATYGKLTLKFICTTGKLPVPWPTLVTTLTYGVQCFSRYPDHMKQHDFFKSAMPEGYIQERTIFFKDDGNYKTRAEVKFEGDTLVNRIELKGIDFKEDGNILGHKLEYN

SEQ ID NO: 6 - protein, 243 aa, synthetic construct
NVYIKADKQKNGIKANFKIRHNIEGGGVQLAYHYQQNTPIGDGPVLLPDNHYLSVQSILSKDPNEKRDHMVLLEFVTAAGITLGMDELYKGGTGGSESMVSKGEELFTGVVPIQVELDGDVNGHKFSVSGEGEGDATYGKLTLKFICTTGKLPVPWPTLVTTLSHGVQCFSRYPDHMKQHDFFKSAMPGGYIQERTIFFKDDGNYKTRAEVKFEGDTLVNRIELKGIDFKEDGNILGHKLEYN

SEQ ID NO: 7 - protein, 242 aa, synthetic construct
VSERMYPEDGALKSEIKKGLRLKDGGHYAAEVKTTYKAKKPVQLPGAYIVDIKLDIVSHNEDYTIVEQCERAEGRHSTGGMDELYKGGTGGSLVSKGEEDNMAIIKEFMRFKVHMEGSVNGHEFEIEGEGEGRPYEAFQTAKLKVTKGGPLPFAWDILSPQFMYGSKAYIKHPADIPDYFKLSFPEGFRWERVMNFEDGGIIHVNQDSSLQDGVFIYKVKLRGTNFPPDGPVMQKKTMGWEA